European Patent Application EP 4 180 056 A1, published May 17, 2023. Title: CMV ANTIGEN AND USES THEREOFF. Applicant: GlaxoSmithKline Biologicals SA. The sequence listing filed with the application follows.

SEQUENCE LISTING (27 sequences)

SEQ ID NO: 1 - protein, 278 aa, Human herpesvirus 5
MCRRPDCGFSFSPGPVILLWCCLLLPIVSSAAVSVAPTAAEKVPAECPELTRRCLLGEVFEGDKYESWLRPLVNVTGRDGPLSQLIRYRPVTPEAANSVLLDEAFLDTLALLYNNPDQLRALLTLLSSDTAPRWMTVMRGYSECGDGSPAVYTCVDDLCRGYDLTRLSYGRSIFTEHVLGFELVPPSLFNVVVAIRNEATRTNRAVRLPVSTAAAPEGITLFYGLYNAVKEFCLRHQLDPPLLRHLDKYYAGLPPELKQTRVNLPAHSRYGPQAVDAR

SEQ ID NO: 2 - protein, 278 aa, Human herpesvirus 5
MCRRPDCGFSFSPGPVALLWCCLLLPIVSSATVSVAPTVAEKVPAECPELTRRCLLGEVFQGDKYESWLRPLVNVTRRDGPLSQLIRYRPVTPEAANSVLLDDAFLDTLALLYNNPDQLRALLTLLSSDTAPRWMTVMRGYSECGDGSPAVYTCVDDLCRGYDLTRLSYGRSIFTEHVLGFELVPPSLFNVVVAIRNEATRTNRAVRLPVSTAAAPEGITLFYGLYNAVKEFCLRHQLDPPLLRHLDKYYAGLPPELKQTRVNLPAHSRYGPQAVDAR

SEQ ID NO: 3 - protein, 278 aa, Human herpesvirus 5
MCRRPDCGFSFSPGPVVLLWCCLLLPIVSSVAVSVAPTAAEKVPAECPELTRRCLLGEVFQGDKYESWLRPLVNVTRRDGPLSQLIRYRPVTPEAANSVLLDDAFLDTLALLYNNPDQLRALLTLLSSDTAPRWMTVMRGYSECGDGSPAVYTCVDDLCRGYDLTRLSYGRSIFTEHVLGFELVPPSLFNVVVAIRNEATRTNRAVRLPVSTAAAPEGITLFYGLYNAVKEFCLRHQLDPPLLRHLDKYYAGLPPELKQTRVNLPAHSRYGPQAVDAR

SEQ ID NO: 4 - protein, 248 aa, Human herpesvirus 5
AAVSVAPTAAEKVPAECPELTRRCLLGEVFEGDKYESWLRPLVNVTGRDGPLSQLIRYRPVTPEAANSVLLDEAFLDTLALLYNNPDQLRALLTLLSSDTAPRWMTVMRGYSECGDGSPAVYTCVDDLCRGYDLTRLSYGRSIFTEHVLGFELVPPSLFNVVVAIRNEATRTNRAVRLPVSTAAAPEGITLFYGLYNAVKEFCLRHQLDPPLLRHLDKYYAGLPPELKQTRVNLPAHSRYGPQAVDAR

SEQ ID NO: 5 - protein, 17 aa, Human herpesvirus 5
GRDGPLSQLIRYRPVTP

SEQ ID NO: 6 - protein, 742 aa, Human herpesvirus 5
MRPGLPSYLIVLAVCLLSHLLSSRYGAEAISEPLDKAFHLLLNTYGRPIRFLRENTTQCTYNSSLRNSTVVRENAISFNFFQSYNQYYVFHMPRCLFAGPLAEQFLNQVDLTETLERYQQRLNTYALVSKDLASYRSFSQQLKAQDSLGEQPTTVPPPIDLSIPHVWMPPQTTPHGWTESHTTSGLHRPHFNQTCILFDGHDLLFSTVTPCLHQGFYLIDELRYVKITLTEDFFVVTVSIDDDTPMLLIFGHLPRVLFKAPYQRDNFILRQTEKHELLVLVKKDQLNRHSYLKDPDFLDAALDFNYLDLSALLRNSFHRYAVDVLKSGRCQMLDRRTVEMAFAYALALFAAARQEEAGAQVSVPRALDRQAALLQIQEFMITCLSQTPPRTTLLLYPTAVDLAKRALWTPNQITDITSLVRLVYILSKQNQQHLIPQWALRQIADFALKLHKTHLASFLSAFARQELYLMGSLVHSMLVHTTERREIFIVETGLCSLAELSHFTQLLAHPHHEYLSDLYTPCSSSGRRDHSLERLTRLFPDATVPTTVPAALSILSTMQPSTLETFPDLFCLPLGESFSALTVSEHVSYVVTNQYLIKGISYPVSTTVVGQSLIITQTDSQTKCELTRNMHTTHSITAALNISLENCAFCQSALLEYDDTQGVINIMYMHDSDDVLFALDPYNEVVVSSPRTHYLMLLKNGTVLEVTDVVVDATDSRLLMMSVYALSAIIGIYLLYRMLKTC

SEQ ID NO: 7 - protein, 6 aa, Human herpesvirus 5
NSVLLD

SEQ ID NO: 8 - protein, 8 aa, synthetic construct
  REGION 1..8: note = source = /note="Description of Artificial Sequence: Synthetic peptide"
DYKDDDDK

SEQ ID NO: 9 - protein, 9 aa, synthetic construct
  REGION 1..9: note = source = /note="Description of Artificial Sequence: Synthetic peptide"
AWRHPQFGG

SEQ ID NO: 10 - protein, 8 aa, synthetic construct
  REGION 1..8: note = source = /note="Description of Artificial Sequence: Synthetic peptide"
WSHPQFEK

SEQ ID NO: 11 - protein, 6 aa, synthetic construct
  REGION 1..6: note = source = /note="Description of Artificial Sequence: Synthetic 6xHis tag"
HHHHHH

SEQ ID NO: 12 - protein, 40 aa, Herpes simplex virus 2
DDVSWRYEAPSVIDYARIDGIFLRYHCPGLDTFLWDRHAQ

SEQ ID NO: 13 - protein, 40 aa, Herpes simplex virus 1
DDLDWRYETPSAINYALIDGIFLRYHCPGLDTVLWDRHAQ

SEQ ID NO: 14 - protein, 39 aa, Varicella zoster virus
EAWDYAAPPVSNLSEALSGIVVKTKCPVPEVILWFKDKQ

SEQ ID NO: 15 - protein, 58 aa, Human herpesvirus 5
EGDKYESWLRPLVNVTGRDGPLSQLIRYRPVTPEAANSVLLDEAFLDTLALLYNNPDQ

SEQ ID NO: 16 - protein, 41 aa, synthetic construct
  REGION 1..41: note = source = /note="Description of Artificial Sequence: Synthetic polypeptide"
EGDKYESWLRPLVNVTEALSGVLLDEAFLDTLALLYNNPDQ

SEQ ID NO: 17 - protein, 48 aa, synthetic construct
  REGION 1..48: note = source = /note="Description of Artificial Sequence: Synthetic polypeptide"
EGDKYESWLRPLVNVTGRDGPLSEALSGVLLDEAFLDTLALLYNNPDQ

SEQ ID NO: 18 - protein, 58 aa, synthetic construct
  REGION 1..58: note = source = /note="Description of Artificial Sequence: Synthetic polypeptide"
EGDKYESWLRPLVNVTGRDGPLSQLIRYRPVTPEALSGVLLDEAFLDTLALLYNNPDQ

SEQ ID NO: 19 - protein, 57 aa, synthetic construct
  REGION 1..57: note = source = /note="Description of Artificial Sequence: Synthetic polypeptide"
EGDKYESWLRPLVNVTGRDGPLSQLIRYRPVTPEAASVLLDEAFLDTLALLYNNPDQ

SEQ ID NO: 20 - protein, 58 aa, synthetic construct
  REGION 1..58: note = source = /note="Description of Artificial Sequence: Synthetic polypeptide"
EGDKYESWLRPLVNVTGRDGPLSQLIRYRPVTPEASSTVLLDEAFLDTLALLYNNPDQ

SEQ ID NO: 21 - protein, 58 aa, synthetic construct
  REGION 1..58: note = source = /note="Description of Artificial Sequence: Synthetic polypeptide"
EGDKYESWLRPLVNVTGRDGPLSQLIRYRPVTPEALSGILLDEAFLDTLALLYNNPDQ

SEQ ID NO: 22 - protein, 58 aa, synthetic construct
  REGION 1..58: note = source = /note="Description of Artificial Sequence: Synthetic polypeptide"
EGDKYESWLRPLVNVTGRDGPLSQLIRYRPVTPEAIEVVLLDEAFLDTLALLYNNPDQ

SEQ ID NO: 23 - protein, 58 aa, synthetic construct
  REGION 1..58: note = source = /note="Description of Artificial Sequence: Synthetic polypeptide"
EGDKYESWLRPLVNVTGRDGPLSQLIRYRPVTPEAIDGVLLDEAFLDTLALLYNNPDQ

SEQ ID NO: 24 - protein, 58 aa, synthetic construct
  REGION 1..58: note = source = /note="Description of Artificial Sequence: Synthetic polypeptide"
EGDKYESWLRPLVNVTGRDGPLSQLIRYRPVTPEALAIVLLDEAFLDTLALLYNNPDQ

SEQ ID NO: 25 - protein, 60 aa, synthetic construct
  REGION 1..60: note = source = /note="Description of Artificial Sequence: Synthetic polypeptide"
EGDKYESWLRPLVNVTGRDGPLSQLIRYRPVTPENLYFQGVLLDEAFLDTLALLYNNPDQ

SEQ ID NO: 26 - protein, 58 aa, synthetic construct
  REGION 1..58: note = source = /note="Description of Artificial Sequence: Synthetic polypeptide"
EGDKYESWLRPLVNVTGRDGPLSQLIRYRPVTPEALSGIVVDEAFLDTLALLYNNPDQ

SEQ ID NO: 27 - protein, 4 aa, Human herpesvirus 5
VTPE